European Patent Application EP 4 397 975 A1, published July 10, 2024. Title: a method of test and a test reagent. Applicant: 国立大学法人京都大学. The sequence listing filed with the application follows.

SEQUENCE LISTING (1 sequence)

SEQ ID NO: 1 - protein, 798 aa, Homo sapiens
METHISVALASNGLYLYSVALALALEUVALTHRGLYALAALAGLNGLYILEGLYARGALAPHEALAGLUALALEULEULEULYSGLYALALYSVALALALEUVALASPTRPASNLEUGLUALAGLYVALGLNCYSLYSALAALALEUASPGLUGLNPHEGLUPROGLNLYSTHRLEUPHEILEGLNCYSASPVALALAASPGLNGLNGLNLEUARGASPTHRPHEARGLYSVALVALASPHISPHEGLYARGLEUASPILELEUVALASNASNALAGLYVALASNASNGLULYSASNTRPGLULYSTHRLEUGLNILEASNLEUVALSERVALILESERGLYTHRTYRLEUGLYLEUASPTYRMETSERLYSGLNASNGLYGLYGLUGLYGLYILEILEILEASNMETSERSERLEUALAGLYLEUMETPROVALALAGLNGLNPROVALTYRCYSALASERLYSHISGLYILEVALGLYPHETHRARGSERALAALALEUALAALAASNLEUMETASNSERGLYVALARGLEUASNALAILECYSPROGLYPHEVALASNTHRALAILELEUGLUSERILEGLULYSGLUGLUASNMETGLYGLNTYRILEGLUTYRLYSASPHISILELYSASPMETILELYSTYRTYRGLYILELEUASPPROPROLEUILEALAASNGLYLEUILETHRLEUILEGLUASPASPALALEUASNGLYALAILEMETLYSILETHRTHRSERLYSGLYILEHISPHEGLNASPTYRASPTHRTHRPROPHEGLNALALYSTHRGLN